European Patent Application EP 4 681 707 A1, published January 21, 2026. Title: Method for treating diseases by using reparixin alone or in combination with Anti-PD-1 antibody. Applicant: SHANDONG CANCER HOSPITAL AFFILIATED TO SHANDONG FIRST MEDICAL UNIVERSITY. Application EP. The sequence listing filed with the application follows.

SEQUENCE LISTING (10 sequences)

SEQ ID NO: 1 - protein, 5 aa, Homo sapiens
SYMMS

SEQ ID NO: 2 - protein, 17 aa, Homo sapiens
TISGGGANTYYPDSVKG

SEQ ID NO: 3 - protein, 7 aa, Homo sapiens
QLYYFDY

SEQ ID NO: 4 - protein, 11 aa, Homo sapiens
LASQTIGTWLT

SEQ ID NO: 5 - protein, 7 aa, Homo sapiens
TATSLAD

SEQ ID NO: 6 - protein, 9 aa, Homo sapiens
QQVYSIPWT

SEQ ID NO: 7 - protein, 443 aa, Homo sapiens
EVQLVESGGGLVQPGGSLRLSCAASGFTFSSYMMSWVRQAPGKGLEWVATISGGGANTYYPDSVKGRFTISRDNAKNSLYLQMNSLRAEDTAVYYCARQLYYFDYWGQGTTVTVSSASTKGPSVFPLAPCSRSTSESTAALGCLVKDYFPEPVTVSWNSGALTSGVHTFPAVLQSSGLYSLSSVVTVPSSSLGTKTYTCNVDHKPSNTKVDKRVESKYGPPCPPCPAPEFLGGPSVFLFPPKPKDTLMISRTPEVTCVVVDVSQEDPEVQFNWYVDGVEVHNAKTKPREEQFNSTYRVVSVLTVLHQDWLNGKEYKCKVSNKGLPSSIEKTISKAKGQPREPQVYTLPPSQEEMTKNQVSLTCLVKGFYPSDIAVEWESNGQPENNYKTTPPVLDSDGSFFLYSRLTVDKSRWQEGNVFSCSVMHEALHNHYTOKSLSLSLGK

SEQ ID NO: 8 - protein, 214 aa, Homo sapiens
DIQMTQSPSSLSASVGDRVTITCLASQTIGTWLTWYQQKPGKAPKLLIYTATSLADGVPSRFSGSGSGTDFTLTISSLQPEDFATYYCQQVYSIPWTFGGGTKVEIKRTVAAPSVFIFPPSDEQLKSGTASVVCLLNNFYPREAKVQWKVDNALQSGNSQESVTEQDSKDSTYSLSSTLTLSKADYEKHKVYACEVTHQGLSSPVTKSFNRGEC

SEQ ID NO: 9 - protein, 116 aa, Homo sapiens
EVQLVESGGGLVQPGGSLRLSCAASGFTFSSYMMSWVRQAPGKGLEWVATISGGGANTYYPDSVKGRFTISRDNAKNSLYLQMNSLRAEDTAVYYCARQLYYFDYWGOGTTVTVSS

SEQ ID NO: 10 - protein, 107 aa, Homo sapiens
DIQMTQSPSSLSASVGDRVTITCLASQTIGTWLTWYQQKPGKAPKLLIYTATSLADGVPSRFSGSGSGTDFTLTISSLQPEDFATYYCQQVYSIPWTFGGGTKVEIK